European Patent Application EP 4 459 280 A1, published November 6, 2024. Title: Screening and uses of glutathione synthetase modulators. Applicant: Max-Planck-Gesellschaft fuer Foerderung der Wissenschaften e.V. Application EP. The sequence listing filed with the application follows.

SEQUENCE LISTING (18 sequences)

SEQ ID NO: 1 - RNA, 20 nt, synthetic construct
  source 1..20: mol_type = other RNA
  misc_feature 1..20: note = CS guide 1 F
caacatggcaagacggtggt

SEQ ID NO: 2 - RNA, 20 nt, synthetic construct
  source 1..20: mol_type = other RNA
  misc_feature 1..20: note = CS guide 1 R
accaccgtcttgccatgttg

SEQ ID NO: 3 - RNA, 20 nt, synthetic construct
  source 1..20: mol_type = other RNA
  misc_feature 1..20: note = CS guide 2 F
ttttccaaaccttaccgtgg

SEQ ID NO: 4 - RNA, 20 nt, synthetic construct
  source 1..20: mol_type = other RNA
  misc_feature 1..20: note = CS guide 2 R
ccacggtaaggtttggaaaa

SEQ ID NO: 5 - RNA, 20 nt, synthetic construct
  source 1..20: mol_type = other RNA
  misc_feature 1..20: note = SLC25A1 guide 1 F
agatctcgatgccacccgcc

SEQ ID NO: 6 - RNA, 20 nt, synthetic construct
  source 1..20: mol_type = other RNA
  misc_feature 1..20: note = SLC25A1 guide 1 R
ggcgggtggcatcgagatct

SEQ ID NO: 7 - RNA, 20 nt, synthetic construct
  source 1..20: mol_type = other RNA
  misc_feature 1..20: note = SLC25A1 guide 2 F
ctacggttccatccccaagg

SEQ ID NO: 8 - RNA, 20 nt, synthetic construct
  source 1..20: mol_type = other RNA
  misc_feature 1..20: note = SLC25A1 guide 2 R
ccttggggatggaaccgtag

SEQ ID NO: 9 - RNA, 25 nt, synthetic construct
  source 1..25: mol_type = other RNA
  misc_feature 1..25: note = AAVS1 F
caccgggggccactagggacaggat

SEQ ID NO: 10 - RNA, 25 nt, synthetic construct
  source 1..25: mol_type = other RNA
  misc_feature 1..25: note = AAVS1 R
aaacatcctgtccctagtggccccc

SEQ ID NO: 11 - DNA, 22 bp, synthetic construct
  source 1..22: mol_type = other DNA
  misc_feature 1..22: note = HMGCR FWD
aggcctgtttgcagatgctagg

SEQ ID NO: 12 - DNA, 20 bp, synthetic construct
  source 1..20: mol_type = other DNA
  misc_feature 1..20: note = HMGCR REV
gatgtcctgctgccaatgct

SEQ ID NO: 13 - DNA, 24 bp, synthetic construct
  source 1..24: mol_type = other DNA
  misc_feature 1..24: note = SQLE FWD
tgggctgctttctgtattgtctcc

SEQ ID NO: 14 - DNA, 22 bp, synthetic construct
  source 1..22: mol_type = other DNA
  misc_feature 1..22: note = SQLE REV
caccactactgagaagggctgg

SEQ ID NO: 15 - DNA, 20 bp, synthetic construct
  source 1..20: mol_type = other DNA
  misc_feature 1..20: note = FDFT1 FWD
ggaaagggcaagcagtgacc

SEQ ID NO: 16 - DNA, 23 bp, synthetic construct
  source 1..23: mol_type = other DNA
  misc_feature 1..23: note = FDFT1 REV
ggatggtggagatgatctgcctt

SEQ ID NO: 17 - DNA, 21 bp, synthetic construct
  source 1..21: mol_type = other DNA
  misc_feature 1..21: note = HPRT1 FWD
tgacactggcaaaacaatgca

SEQ ID NO: 18 - DNA, 21 bp, synthetic construct
  source 1..21: mol_type = other DNA
  misc_feature 1..21: note = HPRT1 REV
cgtccttttcaccagcaagct